European Patent Application EP 4 595 977 A1, published August 6, 2025. Title: Ultra-long-acting platform comprising Fc-advanced fatty acid chain. Applicant: WATERSTONE PHARMACEUTICALS (WUHAN) CO., LTD. The sequence listing filed with the application follows.

SEQUENCE LISTING (17 sequences)

SEQ ID NO: 1 - protein, 275 aa, synthetic construct
HGEGTFTSDVSSYLEEQAAKEFIAWLVKGGGGGGGSGGGGSGGGGSAESKYGPPCPPCPAPEAAGGPSVFLFPPKPKDTLMISRTPEVTCVVVDVSQEDPEVQFNWYVDGVEVHNAKTKPREEQFNSTYRVVSVLTVLHQDWLNGKEYKCKVSNKGLPSSIEKTISKAKGQPREPQVYTLPPSQEEMTKNQVSLTCLVKGFYPSDIAVEWESNGQPENNYKTTPPVLDSDGSFFLYSRLTVDKSRWQEGNVFSCSVMHEALHNHYTQKSLSLSLG

SEQ ID NO: 2 - protein, 5 aa, synthetic construct
TYGMS

SEQ ID NO: 3 - protein, 17 aa, synthetic construct
TISNGGSYTFYPDSVKG

SEQ ID NO: 4 - protein, 11 aa, synthetic construct
HGSVTTRGFDY

SEQ ID NO: 5 - protein, 11 aa, synthetic construct
KASQSVSNDVV

SEQ ID NO: 6 - protein, 7 aa, synthetic construct
YASNRYT

SEQ ID NO: 7 - protein, 9 aa, synthetic construct
LQDYSSPFT

SEQ ID NO: 8 - protein, 445 aa, synthetic construct
EVQLVQSGGGLVQPGGSLKLSCAASGFTFSSYGMSWVRQAPGKGLDWVATISGGGRDTYYPDSVKGRFTISRDNSKNNLYLQMNSLRAEDTALYYCARQKGEAWFAYWGQGTLVTVSSASTKGPSVFPLAPCSRSTSESTAALGCLVKDYFPEPVTVSWNSGALTSGVHTFPAVLQSSGLYSLSSVVTVPSSSLGTKTYTCNVDHKPSNTKVDKRVESKYGPPCPPCPAPEFLGGPSVFLFPPKPKDTLMITRTPEVTCVVVDVSQEDPEVQFNWYVDGVEVHNAKTKPREEQFNSTYRVVSVLTPLHQDWLNGKEYKCKVSNKGLPSSIEKTISKAKGQPREPQVYTLPPSQEEMTKNQVSLTCLVKGFYPSDIAVEWESNGQPENNYKTTPPVLDSDGSFFLYSRLTVDKSRWQEGNVFSCSVMHEALHAHYTQKSLSLSLGK

SEQ ID NO: 9 - protein, 118 aa, synthetic construct
EVQLVQSGGGLVQPGGSLKLSCAASGFTFSSYGMSWVRQAPGKGLDWVATISGGGRDTYYPDSVKGRFTISRDNSKNNLYLQMNSLRAEDTALYYCARQKGEAWFAYWGQGTLVTVSS

SEQ ID NO: 10 - protein, 230 aa, synthetic construct
VESKYGPPCPPCPAPEFLGGPSVFLFPPKPKDTLMITRTPEVTCVVVDVSQEDPEVQFNWYVDGVEVHNAKTKPREEQFNSTYRVVSVLTPLHQDWLNGKEYKCKVSNKGLPSSIEKTISKAKGQPREPQVYTLPPSQEEMTKNQVSLTCLVKGFYPSDIAVEWESNGQPENNYKTTPPVLDSDGSFFLYSRLTVDKSRWQEGNVFSCSVMHEALHAHYTQKSLSLSLGK

SEQ ID NO: 11 - protein, 110 aa, synthetic construct
DIVLTQSPASLAVSPGQRATITCRASESVDNYGISFMNWFQQKPGQPPKLLIYAASNKGTGVPARFSGSGSGTDFTLNINPMEENDTAMYFCQQSKEVPWTFGGGTKLEI

SEQ ID NO: 12 - protein, 218 aa, synthetic construct
DIVLTQSPASLAVSPGQRATITCRASESVDNYGISFMNWFQQKPGQPPKLLIYAASNKGTGVPARFSGSGSGTDFTLNINPMEENDTAMYFCQQSKEVPWTFGGGTKLEIKRTVAAPSVFIFPPSDEQLKSGTASVVCLLNNFYPREAKVQWKVDNALQSGNSQESVTEQDSKDSTYSLSSTLTLSKADYEKHKVYACEVTHQGLSSPVTKSFNRGEC

SEQ ID NO: 13 - protein, 450 aa, synthetic construct
EVQLVQSGSELKKPGASVKVSCKASGYTFTNYGLNWVRQAPGQGLEWMGWINTYTGEPTYADDFKGRFVFSLDTSASTAYLQISSLKAEDMAVYYCAKYGITYEWYFDVWGQGTMVTVSSASTKGPSVFPLAPSSKSTSGGTAALGCLVKDYFPEPVTVSWNSGALTSGVHTFPAVLQSSGLYSLSSVVTVPSSSLGTQTYICNVNHKPSNTKVDKKVEPKSCDKTHTCPPCPAPELLGGPSVFLFPPKPKDTLMISRTPEVTCVVVDVSHEDPEVKFNWYVDGVEVHNAKTKPREEQYNSTYRVVSVLTVLHQDWLNGKEYKCKVSNKALPAPIEKTISKAKGQPREPQVYTLPPSRDELTKNQVSLTCLVKGFYPSDIAVEWESNGQPENNYKTTPPVLDSDGSFFLYSKLTVDKSRWQQGNVFSCSVMHEALHNHYTQKSLSLSPGK

SEQ ID NO: 14 - protein, 214 aa, synthetic construct
DIQMTQSPSSLSASVGDRVTITCRASQDISNSLNWYQQKPGKAPKLLIYYTSRLHSGVPSRFSGSGSGTDFTFTISSLQPEDIATYYCQQGNTFPWTFGSGTKLEIKRTVAAPSVFIFPPSDEQLKSGTASVVCLLNNFYPREAKVQWKVDNALQSGNSQESVTEQDSKDSTYSLSSTLTLSKADYEKHKVYACEVTHQGLSSPVTKSFNRGEC

SEQ ID NO: 15 - protein, 232 aa, synthetic construct
EPKSCDKTHTCPPCPAPELLGGPSVFLFPPKPKDTLMISRTPEVTCVVVDVSHEDPEVKFNWYVDGVEVHNAKTKPREEQYNSTYRVVSVLTVLHQDWLNGKEYKCKVSNKALPAPIEKTISKAKGQPREPQVYTLPPSRDELTKNQVSLTCLVKGFYPSDIAVEWESNGQPENNYKTTPPVLDSDGSFFLYSKLTVDKSRWQQGNVFSCSVMHEALHNHYTQKSLSLSPGK

SEQ ID NO: 16 - protein, 229 aa, synthetic construct
AESKYGPPCPPCPAPEAAGGPSVFLFPPKPKDTLMISRTPEVTCVVVDVSQEDPEVQFNWYVDGVEVHNAKTKPREEQFNSTYRVVSVLTVLHQDWLNGKEYKCKVSNKGLPSSIEKTISKAKGQPREPQVYTLPPSQEEMTKNQVSLTCLVKGFYPSDIAVEWESNGQPENNYKTTPPVLDSDGSFFLYSRLTVDKSRWQEGNVFSCSVMHEALHNHYTQKSLSLSLG

SEQ ID NO: 17 - protein, 15 aa, synthetic construct
GGGGSGGGGSGGGGS